European Patent Specification EP 3 689 895 B1, published July 17, 2024. Title: MODULATION OF SEED VIGOR. Applicant: Syngenta Participations AG. The sequence listing filed with the application follows.

SEQUENCE LISTING (18 sequences)

SEQ ID NO: 1 - DNA, 3061 bp, Brassica oleracea
aaaaagcaggctaagagtgtaagcgacccatttcacatcggatctaaaaatcatataatctagagtctgacaagaatcaacgttgatagagagtgcgagagaatagtacagagccagtcgtcgaggtagaaatgtttgtcctgagcccaaatggtatagttgatattgggattccagaacttgttatcacccactatccatctcttagcggccacctcagtcaccggagctgccgcaagaaaagccagaaccattgccgcagccatcaacgcaagtctagccatagatcactctagaaagaaaaagaagctcagtgcttaatgactcttagtcttatctctcaagaaatagcagttttatgaatgaatgtatatgagcgagtggggctgtttccaagtcaaatcagacatacaaatttctcgttttacggggaaaagatctctcaagatccgtaatttcttcaactaacgtttggaattttattactactttaatcaacctcgatgttgacgatgaagtacacgttaattaaaggtacgcgttatatagttaaaggagtaattagattttaattgctggcattattattatttttctctggtatatttttaaaggaatattttctcaccttttaggcgggaatttatttccattttcttctttcaagggttcagagattcaattcctttattaacatacgaaatgagtatatagtatcttttgaatatttaaataattaaaataaaaataaattaccataacagtgatacatatcaaaatttccaaaactaatgtgagtacttatattagttgtacttcttagtaaaataacgagatatgttatggctcgtcgcatacaacaaagcagagcatatgttcccgcaataacatgcacacgcaactgatagcacgtcgtaaccatttccgcgaaccaaccaatggatattgtaattcgataagacgacgtcgtgttgttgaccacgaatatttcttaaatttccttttatcttttgtttttgacgtcatcacattggtttatgtccacacgatatcagtcataaaatccacgtagggaacgactatccattacacccatccacgtgttctcataacagcttctagttccattagctgaacgaacaatagaaacagagcatcgaactgagaaagaagaagaagaagggaagcaagagaaatggcggcagcggccatggccgttcatctcccgaaacattcatcgtttcttcctaatcccaagcttccattgaatcaaaactctaacttcctcggtgtgtccttgaagatcggtcgacccatgtccgttaaccggaaaatgaaaggtccggttacggtttcagctgcttcgaccgtcgaaggcgatcgaagcaaacagttttacataaacttcactggattcccatttcctcttggtcctttccttaaccggcgcaccatcagaaccgaggttaggctttctccatccctcttgagttttgatttgaactcgttgagaatcccatatggatgttatgcaggcggttaaaggaagcatatggatgtttgaacaagaacaagctttaggtttcagcagtgtctctaccaatataagaatgactgtcatcagactcaaatccggtggcttatgggttcatgcccctattgctcccaccaaagagtgtattcaggttccccctttttattcattatccttgataaagtatcatcctttcttatcatttgataataaccaatgtctaaactcttttttgggttgttttgcaaactttttctttgaggcagcttattgaggagttgggagctccggttgagtacattgtcctgccaacttttgcttacgagcacaagatcttcgtcggtcccttctctagaaagttccccaaggctcaagtatgggtggcgccaagacaatggagctggccactgaacttaccactcgagtttttcggtatctttcgcgctaaaaccattaaagacggagacttatctaccccgtgggctgatgagatcgagcagaaagtcttaagctctcctgaagtcggtacgttccttcactttctcaatcttgttggccctccttagccaagcctcagtgaaacattcgcctaaacccgcactctcctcctcttccctccaaaatatttgaaaagagttatatatacatagcctcccaagttattaaaaaaaacgttttgtctcccaaactattgaaatctttatcaaattgtctatagcctccaaaatccgagggtcggtcctgtacttatgaaataataatatacaggaataggaccgtatgtggaagtagcgttctaccataagcgttcaagaactctattagtcactgatgctgtgatcttcgtcccacggaagccgccatcgagtatcagcagcgagtccttgctggcctctgctaagaacggactggctgtgaagatacttagcaaaggcaaacaagtacctgatgaccctgtcgttgataccccaaacacccgccaaaaaggtcagccatcagcttcttgaaattcaaattcatcaaacaaaagatctcgatgggtgtcttttaacgtgcaggatgggaaagaatggtgctgcaaatcctgtttcttggtccgtctaatctcttggagccaaacgcgagcttcgcacaaatgtcacagaagctgatcgtttctcccattgtcaagactctggtctttagcaaagtccctgagaaggtgagggactggatcgatgagatagcgagtgactggagattcaagaggataatcccagctcatttcgaggctccggtaaacgcagggaggtcagaatttctagctgcgtttgggtttcttgatgatcttctaggggaaagatatgtgaaccgtcctccttcgctctctgttctcttcacttcgctgatgggtaaagcagcgagctattttcctccggatgatatgaggactctctcttctcttgatcagttcttagtctctgttggtgctgttaagaagaccgtctctggtagaaaacgaagatgacggaacaaacccagctttct

SEQ ID NO: 2 - DNA, 5108 bp, Brassica oleracea
gtaggccaagccaagcatatggatcacttagttgagagaagttatggcaagaaataagccatgcagattagaaaaagagtgcaacaaactaagtacagtactaaaagactaagttaataatacaattaaaccaaaattaatggatgagtaccttcacaaaacattagtgaattttcagaccctctggaccaatacaagactaaggatgtgagacttaactgacagttagttcatgtagggccaataaacagctcaaattcgttagctttcaagttccaattttctgcgttgtgttttgctttttgagggttgatttggaatttctccaaagaggtcacataatttaaaagaaattgatcaaaattatattggacaaggcaagcaaatccattaagaagatcacaacaaaagaaaaattaaaaaccaacaaaagaaatttcccatttgacgaaggtgatgaacaagatcagtacgtatactccaccaatgcatgacactactgaaaacatagacaaacaaggtcgtgatagttgtgaccacctcacacatgaaaaaactccatgaatgtcaaaagtttgcacgattatgtaaacacttaatcacttattcattgaaggataatgttggacagaatattatcattgtttctaatggtaagcataagcaaacattgtaaaaagaagtcatgatcatgctatatcttataggagtttaatttattccaagttcacatttagtgatgctctaatcttcaacaataaaacataaccaactgatagtcagagtaaccaattgaatgccagttttcaaaagaaataatacatatctaactgatagtcagtcaaatcaaccaaataagtagaaagaaccaaacaaacacaactaggggtggacacttcgattattttgtaggttcggtttggattcggttcggtttggttaatttattctagaattttttaaactgaagtaaaccataagtttcagtctgatttgtattcggcatggtttgtgtttcagttcagtttaatcggattcccttaatttaattcttttaagaaaaatcatgttttaaaacacggtcatgaaatcatcatgttggtgactatgaaaaaataaattatataattaaatctaatatataactgaaacaaaaatcctaaaaaaccacaaaaaaatttataagaacacaatcaaaccaaagttaactaaagtaaatagaaaattaaaaaaaaaacaatgtcaataaagttaatactgactttagtgttaggatttagtataaaaatgtttaattcaaataataacaaagacacattggtttttcggtgcaatttgattcggttcgattcggttcggtctgatttttttgcttgtctgaacacaacgacggccgacagataactttttaaacgttacgtgaaaatgtattggactattgggccttagtaaaggctaatgaacagattaaatgggcttatagacgcaattgcatggtatctatcgggaagcataaatcgtcaagtaattcaatttaggggactcatttgcaatttgtgcaaagattttagctgtacagagtagggctgaacataaaatccgtaacccgaaatccgaaccgaaccgaaaaacccgatccgtacccgatccaaaatgtaaaaaatacctcaatgaatattgtagggtgttataaaatatatctgaacccgaagtgttattaaccgaacccgaacggataatccgaaaacccgaaaaaccaaaaaattcgaaaaaatatccgaaaaaactgatccgaatgcgtaaattaatataaaatataaatatttgaaacatacattggatatgatatctaacaataagtatttaaaatttaaataaatactttaaatactccattatatacaaagaagtatatattttttatgttttacttttgaattttagattttactatggatatatccgagccgatccgatacaatccgaatccgaatgttatatggctactttggatatatctgaaccgatccgaaaccgaagttgttatatccgaatctcatccgtacttgtaaatttactagaatgagacataggggatgatacaaaatagaaccgaaatccgaaaaaaccgatccgaacccgaacgccgaggcctagtacagagttccgatcagagatagagagaatcctttgagcgtcggccttgctttgtgcgtagggatcatctccgactaattgttgtaattataaagggcggccgcgcctttttagcggagagatggcgagctcacagttcaggtatacgcagacgccgtcgaaggtggtgcacctgaggaatctgccgtgggaatgcgtggaagaggagctcatcgacctatgcaaacgattcggcaagatcgtcaatacgaagaccaatgtcggcgccaatcgcaaccaagcctttgtcgaattcgtaacaactttttattctcttggatcatcagattgtttctttttttggtatctcgttgttgttttggtattgttgttttgaagatgaaactgtatactttgattcatattcgcagggtgacgtgaatcaggcaatatcaatggtttcttactatgcttcgtcttcagagccggctcagattcgagggaagactgtttatattcagtactctaatcgccatgagattgtcaacaatcagagtcctggagaggtccctggcaatgtcctcttggtcacctttgaaggagtccaatctcaccatgtctgcatcgatgtcatccatctggtatgtgaatattcagcttaccttccactattgtttcttgttatgttaagtgatttttttcgtttcttcgagtagattctaatctatgaaaatatttcaacttgttgttattaggcaaacttcttttgagtgtatttttttccacttattgttagacatacagtatgtcacatactattgtaaattacagtatatctgacgttaatgaaaatgctcgaatcacagatgttgatgcctctttattataatctttctggagagagtttggaaaatagtttcatgttcgtcattctcatggacaggtgtcactctgcacttatctagtcattctcttttttagtctcctaatttgagtttatttcgattgatttgcttcccttagttattatcaatttactccactgtattatatggacatgactcatatctagtccaaacttttgtttcaggtgttttctgcttatggcttcgtgcacaaaattgccacttttgagaaagctgctggtttccaggttagagatatcgagttttgttttcaaggtcttgcataaatctaatgatgtttaaactcatcgtctgccgtcataacctgctcaggcacttgttcagtttactgatgtggacactgccttagcggcaaggactgcgctggatggtagaagtatacccaagtatgctcaaatccttcattcatgcttttgaccataagataaagctctgttgatggtttcttccttttcttttggtaaattcagatatctgcttccagaacatgtaggctcatgcaatttgcgaatgtcttactcagctcatactgatctaaatatcaaatttcagtcccaccgcagcaggtagagttttgagtcctcgcaaatgtgcctctccattgttatactgctcttactgttggaagccttatggttgaatagttacttcatgtgtttaattctcttacgcactcagggactacacaaatccataccttccggtgaatcaaaccgctatggacggttctatgcaggtatatttttcctttgatctaatcttatctccaacagcttatattattcttacactgaatgcgtttgtattacgttactgatcgtctttgtccatcactgcgttcagcctgctttgggtgctgatggaaagagggttgaaactcagagcaacgtcctgcttgctttgattgagaatatgcagtacgctgtcaccgtggatgttcttcacacggtgaggaacaacaatatgcctgtttcttcatctcatcatgctttcatatctcaaaattaactattcctttgcttctcataggtgttttccgcttatggaactgtgcagaagattgcaatatttgagaaaaatggttcaacgcaagccttaattcaatactctggtacatgaccttgataatctgaatacatatatgattctactatacttcttttggttatatggtgaatcttcttatgtgtatgcaaagagaagagcctaagaatttgaatatagtcatcgtttgcttcatgttccgttttattgattcttctgtagacatttcaacggcgacgatggcgaaagaagcactggagggacactgcatatatgacggaggctactgtaagcttcgactaacttactctcggcatactgatctcaatgtaaaggtacataagatcagttgctttatgtacccaaacaaaaagtgcagttaaagagaataagaagtgatttctgcaagaaccgcatgcttttttctcatcaacaattgagtgaaatctgaattcgacattctagttgattcaactaatgattttcgtcttctttcttcaggcatttagcgacaaaagcagagactacacactgcctgatctaagccaactggtgggccaaaaggttccaggagtggctgcagctagtgggccaacagatggttggcccaatgggcaggtgcagactcaatacatgggaagttcgtatatgtacccaccagctgatcccacaggagcttcaccttcttctggtcatcctccttattatggttgatccatgtactgttttctactttatataaatttcggattatgttgaagactagtttccatgttataggtttcaggtaaaagtgtgttgttcttttatttggttaaataaacatgggaaaaccaataatattatgtagtataatttataaacattgtgtatttgtttctatttgactttgttatggagcttccgaagtgttagagcttctttttctcgtactttaaactgtttcattcctggatttgtttgaagatctgcagacttacactttagtgacttttggtatcc

SEQ ID NO: 3 - DNA, 3025 bp, Brassica oleracea
aaaaagcaggctaagagtgtaagcgacccatttcacattggatctaaaaatcaaataatctagagtgtgacaagaatcaacgttgatagagagtgagagagaatagtacagagccagtcgtcgaggtagaaatgtttgtcctgagcccaaatggtatagttgatattgggattccagaacttgttatcacccactatccatctcttagcggccacctcagtcaccggagctgccgcaagaaaagccagaaccactgccgcagccatcaacgcaagtctagccatagatcactctagaaagaaaaagaagctcagtgcttgatgactcttagtcttatctctcaagaaatagcagttttatgagtgagtggggctgtttccaagtcaaatcagacatacaaatttctcgttttacggggaaaagatctctcaagatccgtaatttcttcaactaacgtttggaatcttattactactttaatcaacctcgatgttgacgatgacgtacacgttaattaaaggtacgcgttatatagttaagggagtaattagattttaactgctggcattattattatttttctctggttattacattattctgttttgtagtaatattttctcaccttttaggcgggaatttatttccattttcttctttcaagggttcagagattcaattcctttattaacatacgaaatgagtatatagtatcttttaaatatttaaataattaaaataaaaataaattactataacagtgatacatatcaaaatttccaaaactaatgtgagtacttatattagttgtacttcttagtaaaataacgagatatgttatggctcgtcgcatacagcaaagcagagcatatgttcccgcaataacatgcacacgcaactgatagcacgtcgtaaccatttccgcgaaccaaccaatggatattgtaattcgataagacgacgtcgtgttgttgaccacgaatatttcttaaatttccttttatcttttgtttttgacgtcatgacattggtttatgtccacacgatatcagtcataaaatccacgtaggaacgactatccattacacccatccacgtgttctcataacagcttctagttccattagctgaacgaacaatagaaacagagcatcgaactgagaaagaagaagaagaagggaagcaagagaaatggcggcagcggccatggccgttcatctcccgaaacattcatcgtttcttacgaaacccaagcatccatccgatcaaaactctaactttctcggtgggtccttaaagttcggtcgatccatgtctctaaaccggaaaactaaaggtccagttatggtttcagctgcttcgaccgtcgaaggcgatcgaagcaaacagttttacataaacttcactggattcccatttcctcttggtcctttccttaaccggcgcaccatcagaaccgaggttaggctttctccatccctcttgagttttgatttgaactcgttgagaatcccatatggataatgttatgcaggcggttaaaggaagcatatggatgtttgaacaagaacaagctttaggtttcagcagtgtctcaacgaatataagaatgactgtcatcaaactcaaatccggtggcttatgggttcatgcccctattgctcccaccaaagagtgtattcaggttccctcttttattcattatcagtatcatcctttcttatcatttgataaattaaccaatgtctaaactctattttgggttgttttgcttactttttctttggggcagcttattgaggagttgggagctccggttgagtacatcgtcctaccaaccttcgcttacgagcacaagatcttcgtcggtcccttctctagaaagttccccaaggctcaagtatgggtggcgccaagacaatggagctggccactgaacttaccactcgagtttttcggtatctttcgcgctaaaaccattaaagacggtgacttgtctaccccgtgggctgatgagatcgagcagaaagtcttaagctctcctgaagtcggtacgttccttcactttctcaatcttgttggccctccttagccaagcctcataaaacattcgcttcaacccctcaccccacccaaattttttgaaaaaagttacatatacatagccccaaatttattaaaaaaatctattgaaatctttattaaattatctacgtcccctagaatctgagggtcggccctgtacttatggaataaataatatacaggaattggaccgtatgtggaagtagcgttctaccataagcgttcaagaactctattagtcaccgacgctgtgatcttcgtcccaaagaagccgccatcgagtatcagcagcgagtctttgctggcttctgctaagaacggactggctgtgaagatacttagcaaaggcaaacaagtacctaatgaccctgtcgttgataccccaaacacccgccaaaaaggtcagccatcagcttcttgaaattcaaattcatcaaacaaagatctcaatgggtgtcttttaacgtgcaggatgggaaagaatggtgctgcaaatcctgtttctcggcccatctaatctcttggagccaaacgcgagctttgcgcaaatgtcacagaagctgatagtttctcccattgtcaagactctggtctttagcaaagtccctgagaaggtgagggactggatcgatgagatagcgagtgactggaggttcaagaggataatcccagctcatttcgaggctccgataaacgcggggaggtcagagtttctagctgcgttcgggtttcttgatgatcttctaggggaaagatatgtgaaccgtcctccttcgctctctgttctctttacttcgctgatgggtaaagctgccagctattttcctccggatgatatgagaactctctcttctcttgatcagttcttagtctctgttggtgctgttaagaagaccgtctctggtagaaaacgaagatgacggaacaaacccagctttct

SEQ ID NO: 4 - DNA, 4992 bp, Brassica oleracea
gtaggccaagccaagcatatggatcacttagttgagagaagttatggcaagaaataagccatgcagattagaaaaagagtgcaacaaactaagtacagtactaaaagactaagttaataatacaattaaaccaaaattaatggatgagtaccttcacaaaacattagtgaattttcagaccctctggaccaatacaagactaaggatgtgagacttaactgacagttagttcatgtagggccaataaacagctcaaattcgttagctttcaagttccaattttctgcgttgtgttttgctttttgagggttgatttggaatttctccaaagaggtcacataatttaaaagaaattgatcaaaattatattggacaaggcaagcaaatccattaagaagatcacaacaaaagaaaaataaaaaaccaacaaaagaaatttcccatttgacgaaggtgatgaacaagatcagtacgtatactccaccaatgcatgacactactgaaaacatagacaaacaaggtcgtgatagttgtgaccacctcacacatgaaaaaactccatgaatgtcaaaagtttgcacgattatgtaaacacttaatcacttattcattgaaggataatgttggacagaatattatcattgtttctaatggtaagcataagcaaacattgtaaaaagaagtcatgatcatgctgtatcttataggagtttaatttattccaagttcacatttagtgatgctctaatcttcaacaataaaacataaccaactgatagtcagagtaaccaattgaatgccagttttcaaaagaaataatacatatctaactgatagtcagtcaaatcaaccaaataagtagaaagaaccaaacaaacacaactagggtggacacttcgattattttgtaggttcggtttggattcggttcggtttggttaatttattctagaatttttttaactgaagtaaaccataagtttcagtctgatttgtattcggcatggtttgtgtttcagttcagtttaatcggattcccttaatttaattcttttaagaaaaatcatgttttaaaacatggtcatgaaatcatcatgttggttactatgaaaaaataaattatataattaaatctaatatataactgaaacaaaaatcctaaaaaaccacaaaaaattttataagaacacaatcaaaccaaagttaactaaagtaaatagaaaattaaaaaaaaaaacaatgtcaataaagttaatactgactttagtgttaggatttagtataaaaatgtttaattcaaataataacaaaaacacattggtttttcggtgcaatttgttcggtttgattcggttcggtctgatttttttgcttctctgaacacaacgacggccgacagataactttttaaacgttacgtgaaaatgtattggactattgggccttagtaaaggctaatgaacagattaaatgggcttatagacgcaattgcatggtatctatcgggaagcataaatcgtcaagtaattcaatttaggggactcatttgcaatttgtgcaaagattttagctgtacagagtagggctgggcataaaatccgtaacccgaaatccgaaccgaaccgaaaaacccgatccgtacccgatccaaaatgtaaaaaatacctcaatggatattgtagggtgttataaaatatatctgaacccgaagtgttattaaccgaacccgaacggataatccgaaaacccgaaaaaccaaaaaactcgaaaaaatatccgaaaaaactgatccgaatgcgtaaattaatataaaatataaatatttgaaacatacattggatatgatatctaacaataagtatttaaaatttaaataagtactttaaatactctattatatacaaagaagtatatattttttatgttttacttttgaattttagattttactatgtatatatccgagccgatccgatacaatccgaatccgaatgttatatggctattttggatatatctgaaccgatccgaaaccgaagttgttatatccgaatctcatccgtactggtaaatttactagaatgagacacgggggatgatacaaaatagaaccgaaatccgaaaaaaccgatccgaaccgaacgcccaggcctagtacagagttccgatcagagatagagagaatcctttgagcgtcggccttgctttgtgcgtagggatcatctccgactaattgttgtaattataaagggcggccgcgcctttttagcggagagatggcgagctcacagttcaggtatacgcagacgccgtcgaaggtggtgcacctgaggaatctgccgtgggaatgcgtggaagaggagctcatcgacctatgcaaacgattcggcaagatcgtcaatacgaagaccaatgtcggcgccaatcgcaaccaagcctttgtcgaattcgtaacaactttttattctcttcgatcatcagattgtttctgaagctttgtgatttctatgatgaactcttttttttttggtatctcgttgttgttttggtattgttgttttgaagatgaaactgtatactttgattcatattcgcagggtgacgtgaatcaggcaatatcaatggtttcttattatgcttcgtcttcagagccggctcagattcgagggaagactgtttatattcagtactctaatcggcatgagattgtcaacaatcagagtcctggagaggtccctggcaatgtcctcttggtcacctttgaaggagtccaatctcaccatgtctgcatcgatgtcatccatctggtatgtgaatattcagcttaccttccactattgtttcttgttatgttaagtgatttttttcgtttcttcgagtagattctaatctatgaaaatatttcaacttgttgttattaggcaaacttcttttgagtgtatttttttccagttattgttagacatacagtatgtcacatactattgtaaattacagtatatctgacgttaatgaaaatgctcgaatcacagatgttgatgcctctttattataatctttctggagagagtttggaaaatagtttcatgttcgtcattctcatggacaggtgtcactctgcacttatctagtcattctcttttttagtctcctaacccggcaacatttgagtttatttcgattgatttgcttcccttagttattatcaatttactccactgtattatatggacatggctcatatctagtccaaacttttgtttcaggtgttttctgcttatggcttcgtgcacaaaattgccacttttgagaaagctgctggtttccaggttagagatatcgagttttgttttcaaggtcttgcctaaatctaatgatgtttaaactcatcgtctgccgtcataacctgctcaggcacttgttcagtttactgatgtggacactgccttagcggcaaggactgcgctggatggtagaagtatacccaagtatgctcaaatccttcattcatgcttttgaccataagataaagctctgttgatggtttcttccttttcttttggtaaattcagatatctgcttccagaacatgtaggctcatgcaatttgcgaatgtcttactcagctcatactgatctaaatatcaaatttcagtcccaccgcagcaggtagagttttgagtcctcgcaaatgtgcctctccattgttatactgctcttactgttggaagccttatggttgaatagttacttcatgtgtttaattctcttacgcactcagggactacacaaatccataccttccggtgaatcaaaccgctatggacggttctatgcaggtatatttttcctttgatctaatcttatctccaacagcttatattattcttacactgaatgcgtttgtattacgttactgatcgtctttgtccatcactgcgttcagcctgctttgggtgctgatggaaagagggttgaaactcagagcaacgtcctgcttgctttgattgagaatatgcagtacgctgtcaccgtggatgttcttcacacggtgaggaacaacaatatgcctgtttcttcatctcatcatgctttcatatctcaaaattaactattcctttgcttctcataggtgttttccgcttatggaactgtgcagaagattgcaatatttgagaaaaatggttcaacgcaagccttaattcaatactctggtacatgaccttgataatctgaatacatatatgattctactatacttcttttggttatatggtgaatcttcttatgtgtatgcaaagagaagagcctaagaatttgaatatagtcatcgtttgcttcatgttccgttttattgattcttctgtagacatttcaacggcgacgatggcgaaagaagcactggagggacactgcatatatgacggaggctactgtaagcttcgactaacttactctcggcatactgatctcaatgtaaaggtacataagatcagttgctttatgtacccaaacaaaaagtgcagtcaaagagaataataagtgatgtctgcaagaaccgcatgcttttttctcatcaacaattgagtgaaatctgaattcgacattctagttgattcaactaatgattttcgtcttctttcttcaggcatttagcgacaaaagcagagactacacactgcctgatctaagccaactggtgggccaaaaggttccaggagtggctgcagctagtgggccaacagatggttggcccaatgggcaggtgcagactcaatacatgggaagttcgtatatgtacccaccagctgatcccacaggagcttcaccttcttctggtcatcctccttattatggttgatccatgtactgttttctactttatataaatttcggattatgttgaagactagtttccatgttataggtttcaggtaaaagtgtgttgttcttttatttggttaaataaacatgggaaaaccaataatattat

SEQ ID NO: 5 - DNA, 4993 bp, Brassica oleracea
acgtctatgaccggagtagtctccttcgtgaagaccggtcactgaaacgcgaatgatgttcgccataatctcccatttctttgaaggtatttgaacggtttggtgggttgattgaggcggatcttaagcagctcgagtggatctaatcagctgagagaatcggggagacgattagatcatgcggtgacagattcgagaggaaaccctaatcgccatcgccgccagagagtctcatgtgcagtgtgattcatatgcaaatctcgtggatttggttgtttttttctttttcaggtttgatttggaatttctctaaagaggtcacattaattaaaataaactagacccttatccgcgcgccagcgcagatatgaatttttagtttttaattatttattttattcaatgatgtatttgtaatattcgttcatattatattcgttaagtaaatatttttttgtatcttaaactatctatttttttacgaatgtgtgatatcatataaaaatattaaaaaatgagtatagagttaataagataattttaaaaacagaaatttttctttcgtgtgcgatatcatataaataatgatccgcccagttaacaaaaatcatgattattttatgtgtaattttctttattttgactatttccttaaaactatattaaattttacatattttaattagaatatttttaatatctttacctttttatttgaaatgcaactcaatatttttttttaacaattataacaaaatatttaaaaaatatttttagaatttgtttgaaaaatatgaaaattacattttaaattaaaattatcctaaaatatgataagttttgatgtaaacgaaaactcaaattatgtcaaaaataatgatattcaatgataataacaattttaattgattattttttaaaaaatacatttacaaaaatattgtttgaaagaaaattcatttatctttcaaatataaaatgaaaatattataattaaataataaaaaatataaataaaaaccataaatttagcaaatgacaactgagttatattatgctaaaaaaaaatttctaacaaaatatcaaatgacaaatgagttatgagtaaataataccatataatttttaaaaacatagccattcttaaatattttttgaataaataattattttaaatttaatcaactaaaaataatatctgtacaattgtgtgagtcaaattctagttttattgatgcatgttatatattagtgctgcatgttttaggtaacattttaatgatgcacgttttcaaaaatctccattattaaaattatgcacgtaatgataactcatgagttttttttgttgattaaatgacattatgtccaaatttatttaaggatatttcattaaggtaagtgaaaaagacaaacaataaaataggaagtttaaaatcatttaagcatatttcattaatgtaactgaaaagacaagtaataaattaggcagttttattcgttttatgatatttcataaatgcaactggaaaagacaaacaaaaaaaaatagggagtttaattaatgaaataagaacattttcaaatgagtacttctcttttaataatatagatttcattaatgtaactgaaaagacaagtaataaattaggcagttttattcgttttagtatatttcataaatgcaactgaaaaagacaagaaaaaaaaataaagaatttaattaatgaagtaagaatattttcaaatgagtatttctcttttaataatatagattgatcaaaaattatattggataaggcaagcaaaatccattgagaagatcacaacaacaaaagaaaggaacaaacacacaaccacggcgacagataactaaaatgtactggactattgggcccttaatataggctaatgaacagattaaatgggctaattatagacgtcattgcatggtatccatctatctggaagcatagtaatttgttttaggggactggtttgcaatttttacagatattttagctgtacagtacagagagagaatcctttgagcgtcgtcggccttgctttgtgtgtagggatctccgactgactaattgttgtaactacaaaagggcgccccccgcgcctttttactagatggcgagctcatcacagtttaggtatacccagacgccgtcgaaggtggtgcacctgaggaatctgccgtgggaatgcgtggaagaggagctcatcgacctatgcaaacgattcggcaagatcgtcaatacgaagaccaatgtcggcgccaatcgcaaccaagcctttgtcgaattcgtaagaactttttattctcttggatcatcagattgttgcttcccccccaatggatttggttagaaattgaataaaaaaaggactcgaactctttttttggtatctcgttgttgttttgaagatgaaactgtatactttgattcatattcgcagggtgacgtgaatcaggcaatatcaatggtttcttactatgcttcgtcttcagagccggctcagattcgagggaagactgtttatattcagtactctaatcgccatgagattgtcaacaatcagagtcctggagaggtccctggcaatgtcctattggtcacctttgaaggagtccaatctcaccatgtctgcatcgatgtcatccatctggtatgtgaatattcagcttaccttccactattgtttcttgttatagtgatttttttcgtttcttcgagtagattctaatctatgaaaatatttcaacttgttgttattaggcaaacttcttttgagtgtatttttttccagttattgttagacatacagtatgtcacatactattgtaaattacagtatatctgacgttaatgaaaatgctcgaatcacagatgttgatgcctctttattataatctttctggagagagtttggaaaatagtttcatgttcgtctttctcatggacaggtgtcactctgcacttatctagtcattctcttttttagtctcctaatttgagtttatttcgattgatttgcttcccttagttattatcaatttactccactgtattatatggacatgactcatatctagtccaaacttttgtttcaggtgttttctgcttatggcttcgtgcacaaaattgccacttttgagaaagctgctggtttccaggttagagatatcgagttttgttttcaaggtcttgcctttttcataaaatctaatgatgtttaaactcatcatctgccgtcataacctgctcaggcacttgttcagtttactgatgtggacactgccttagcggcaaggactgcgctggatggtagaagtatacccacgtatgctcaaatccttcattcatgcttttgaccataagataaagctctgttgatggtttcttccttttcttttggtaaattcagatatctgcttccagaacatgtaggctcatgcaatttgcgaatgtcttactcagcccacactgatctaaatatcaaatttcagtcccaccgcagcaggtagagttttgagtcctcgcaaatgtgccattccattgttttactgctcctactgttggaagccttatggttgaatagttgattcatgtgttttgattttctgacgtactcagggactacacaaatccatatcttccggtgaatcaaactgctatggatggttctatgcaggtaaatatttcctctttctagtctatctccaacagcttagacaattcttacattgaatgcgttactgattgtctttgacgtcattgcattcagcctgctttgggtgctgatggaaagagggtagaaactcagagcaacgtcctacttgctttgattgagaatatgcaatacgctgtcacacggtgaggaacaccattatgcacgtttctgcatctcagcatcctttcatttctcaaaattaattatttcctttgcttgtcataggtgttttccgcttatgggactgtgcagaagattgcaatatttgagaaaaatggttcaacgcaagccttaattcaatactctggtacatgaccttgatgatctgaatacatatattattatactatacttctttcggttatatggcgaatcatcttatgtgtatgctaagaatttgaatagtcatcatttgcttcatgttccgttttcttgattcttctgtagacataccaacggcgacaatagcgaaagaagcattggagggacactgcatatatgacgggaggctactgtaagcttcgactaacatactcgtcatactgatctcaatgtaaaggtacgtaagatcagttgctttcttgatttgtgcacccaaacaaaaaagcttggggaaagagaataataacttatgtctgcaagaaccatatgctattttttttctcttcaacaattgtatgaaatctgaattcgactttctagtttattcaactagtgatttttcgtcttctttcttcaggcatttagtgacaaaagcggagactacacactgcctgatctaagccaactggtgggccaaaaggttccaggagtggccgctgctagtgggccaacagattgttggcacaatgggcaggtgcagactcaatacacaagaagttcatatatgtacccactgtaagcaaaggtactagattttgataaagcgcgagtttatttttaaatttttttcaattgacaaatatttagtaaatgtcatattttcatatatttgtgttttattttataaaagacttaaactttttatctttatttatcgtattttattttaaatgactatttatgtttaaaaaattaaactttatttctttaatgaattaagttgatataactctgataaattaattttattatgtggttaatattttaattaaaaaaaattatatacttttaataaagatttgtatttttcaatgaaaaaattcaattttttttatgaatgcttaaattatattaagaaaagaaaaga

SEQ ID NO: 6 - DNA, 4992 bp, Brassica oleracea
acgtctatgaccggagtagtctccttcgtgaagaccggtcactgaaacgcgaatgatgttcgccataatctcccatttctttgaaggtatttgaacggtttggtgggttgattgaggcggatcttaagcagctcgagtggatctaatcagctgagagaatcggggagacgattagatcatgcggtgacagattcgagaggaaaccctaatcgccatcgccgccagagagtctcatgtgcagtgtgattcatatgcaaatctcgtggatttggttgtttttttctttttcaggtttgatttggaatttctctaaagaggtcacattaattaaaataaactagacccttatccgcgcgccagcgcagatatgaatttttagtttttaattatttattttattcaatgatgtatttgtaatattcgttcatattatattcgttaagtaaatatttttttgtatcttaaactatctatttttttacgaatgtgtgatatcatataaaaatattaaaaaatgagtatagagttaataagataattttaaaaacagaaatttttctttcgtgtgcgatatcatataaataatgatccgcccagttaacaaaaatcatgattattttatgtgtaattttctttattttgactatttccttaaaactatattaaattttacatattttaattagaatatttttaatatctttacctttttatttgaaatgcaactcaatattttttttaacaattataacaaaatatttaaaaaatatttttagaatttgtttgaaaaatatgaaaattacattttaaattaaaattatcctaaaatatgataagttttgatgtaaacgaaaactcaaattatgtcaaaaataatgatattcaatgataataacaattttaattgattattttttaaaaaatacatttacaaaaatattgtttgaaagaaaattcatttatctttcaaatataaaatgaaaatattataattaaataataaaaaatataaataaaaaccataaatttagcaaatgacaactgagttatattatgctaaaaaaaaatttctaacaaaatatcaaatgacaaatgagttatgagtaaataataccatataatttttaaaaacatagccattcttaaatattttttgaataaataattattttaaatttaatcaactaaaaataatatctgtacaattgtgtgagtcaaattctagttttattgatgcatgttatatattagtgctgcatgttttaggtaacattttaatgatgcacgttttcaaaaatctccattattaaaattatgcacgtaatgataactcatgagttttttttgttgattaaatgacattatgtccaaatttatttaaggatatttcattaaggtaagtgaaaaagacaaacaataaaataggaagtttaaaatcatttaagcatatttcattaatgtaactgaaaagacaagtaataaattaggcagttttattcgttttatgatatttcataaatgcaactggaaaagacaaacaaaaaaaaatagggagtttaattaatgaaataagaacattttcaaatgagtacttctcttttaataatatagatttcattaatgtaactgaaaagacaagtaataaattaggcagttttattcgttttaggatatttcataaatgcaactgaaaaagacaagaaaaaaaaataaagaatttaattaatgaagtaagaatattttcaaatgagtacttctcttttaataatatagattgatcaaaaattatattggataaggcaagcaaaatccattgagaagatcacaacaacaaaagaaaggaacaaacacacaaccacggcgacagataactaaaatgtactggactattgggcccttaatataggctaatgaacagattaaatgggctaattatagacgtcattgcatggtatccatctatctggaagcatagtaatttgttttaggggactggtttgcaatttttacagatattttagctgtacagtacagagagagaatcctttgagcgtcgtcggccttgctttgtgtgtagggatctccgactgactaattgttgtaactacaaaagggcgccccccgcgcctttttactagatggcgagctcatcacagtttaggtatacccagacgccgtcgaaggtggtgcacctgaggaatctgccgtgggaatgcgtggaagaggagctcatcgacctatgcaaacgattcggcaagatcgtcaatacgaagaccaatgtcggcgccaatcgcaaccaagcctttgtcgaattcgtaacaactttttattctcttggatcatcagattgttgcttcccccccaatggatttggttagaaattgaataaaaaaaggactcgaactctttttttggtatctcgttgttgttttgaagatgaaactgtatactttgattcatattcgcagggtgacgtgaatcaggcaatatcaatggtttcttactatgcttcgtcttcagagccggctcagattcgagggaagactgtttatattcagtactctaatcgccatgagattgtcaacaatcagagtcctggagaggtccctggcaatgtcctattggtcacctttgaaggagtccaatctcaccatgtctgcatcgatgtcatccatctggtatgtgaatattcagcttaccttccactattgtttcttgttatagtgatttttttcgtttcttcgagtagattctaatctatgaaaatatttcaacttgttgttattaggcaaacttcttttgagtgtatttttttccagttattgttagacatacagtatgtcacatactattgtaaattacagtatatctgacgttaatgaaaatgctcgaatcacagatgttgatgcctctttattataatctttctggagagagtttggaaaatagtttcatgttcgtctttctcatggacaggtgtcactctgcacttatctagtcattctcttttttagtctcctaatttgagtttatttcgattgatttgcttcccttagttattatcaatttactccactgtattatatggacatgactcatatctagtccaaacttttgtttcaggtgttttctgcttatggcttcgtgcacaaaattgccacttttgagaaagctgctggtttccaggttagagatatcgagttttgttttcaaggtcttgcctttttcataaaatctaatgatgtttaaactcatcatctgccgtcataacctgctcaggcacttgttcagtttactgatgtggacactgccttagcggcaaggactgcgctggatggtagaagtatacccacgtatgctcaaatccttcattcatgcttttgaccataagataaagctctgttgatggtttcttccttttcttttggtaaattcagatatctgcttccagaacatgtaggctcatgcaatttgcgaatgtcttactcagcccacactgatctaaatatcaaatttcagtcccaccgcagcaggtagagttttgagtcctcgcaaatgtgccattccattgttttactgctcctactgttggaagccttatggttgaatagttgattcatgtgttttgattttctgacgtactcagggactacacaaatccatatcttccggtgaatcaaactgctatggatggttctatgcaggtaaatatttcctctttctagtctatctccaacagcttagacaattcttacattgaatgcgttactgattgtctttgacgtcattgcattcagcctgctttgggtgctgatggaaagagggtagaaactcagagcaacgtcctacttgctttgattgagaatatgcaatacgctgtcacacggtgaggaacaccattatgcacgtttctgcatctcagcatcctttcatttctcaaaattaattatttcctttgcttgtcataggtgttttccgcttatgggactgtgcagaagattgcaatatttgagaaaaatggttcaacgcaagccttaattcaatactctggtacatgaccttgatgatctgaatacatatattattatactatacttctttcggttatatggcgaatcatcttatgtgtatgctaagaatttgaatagtcatcatttgcttcatgttccgttttcttgattcttctgtagacataccaacggcgacaatagcgaaagaagcattggagggacactgcatatatgacgggaggctactgtaagcttcgactaacatactcgtcatactgatctcaatgtaaaggtacgtaagatcagttgctttcttgatttgtgcacccaaacaaaaaagcttggggaaagagaataataacttatgtctgcaagaaccatatgctattttttttctcttcaacaattgtatgaaatctgaattcgactttctagtttattcaactagtgatttttcgtcttctttcttcaggcatttagcgacaaaagcggagactacacactgcctgatctaagccaactggtgggccaaaaggttccaggagtggccgctgctagtgggccaacagattgttggcacaatgggcaggtgcagactcaatacacaagaagttcatatatgtacccactgtaagcaaaggtactagattttgataaagcgcgagtttatttttaattttttttcaattgacaaatatttagtaaatgtcatattttcatatatttgtgttttattttataaaagacttaaactttttatctttatttatcgtattttattttaaatgactatttatgtttaaaaaattaaactttatttctttaatgaattaagttgatataactctgataaattaattttattatgtggttaatattttaattaaaaaaaattatatacttttaataaagatttgtatttttcaatgaaaaaattcaattttttttatgaatgcttaaattatattaagaaaagaaaaga

SEQ ID NO: 7 - protein, 448 aa, Brassica oleracea
MAAAAMAVHLPKHSSFLPNPKLPLNQNSNFLGVSLKIGRPMSVNRKMKGPVTVSAASTVEGDRSKQFYINFTGFPFPLGPFLNRRTIRTEAVKGSIWMFEQEQALGFSSVSTNIRMTVIRLKSGGLWVHAPIAPTKECIQLIEELGAPVEYIVLPTFAYEHKIFVGPFSRKFPKAQVWVAPRQWSWPLNLPLEFFGIFRAKTIKDGDLSTPWADEIEQKVLSSPEVGIGPYVEVAFYHKRSRTLLVTDAVIFVPRKPPSSISSESLLASAKNGLAVKILSKGKQVPDDPVVDTPNTRQKGWERMVLQILFLGPSNLLEPNASFAQMSQKLIVSPIVKTLVFSKVPEKVRDWIDEIASDWRFKRIIPAHFEAPVNAGRSEFLAAFGFLDDLLGERYVNRPPSLSVLFTSLMGKAASYFPPDDMRTLSSLDQFLVSVGAVKKTVSGRKRR

SEQ ID NO: 8 - protein, 395 aa, Brassica oleracea
MASSQFRYTQTPSKVVHLRNLPWECVEEELIDLCKRFGKIVNTKTNVGANRNQAFVEFGDVNQAISMVSYYASSSEPAQIRGKTVYIQYSNRHEIVNNQSPGEVPGNVLLVTFEGVQSHHVCIDVIHLVFSAYGFVHKIATFEKAAGFQALVQFTDVDTALAARTALDGRSIPKYLLPEHVGSCNLRMSYSAHTDLNIKFQSHRSRDYTNPYLPVNQTAMDGSMQPALGADGKRVETQSNVLLALIENMQYAVTVDVLHTVFSAYGTVQKIAIFEKNGSTQALIQYSDISTATMAKEALEGHCIYDGGYCKLRLTYSRHTDLNVKAFSDKSRDYTLPDLSQLVGQKVPGVAAASGPTDGWPNGQVQTQYMGSSYMYPPADPTGASPSSGHPPYYG

SEQ ID NO: 9 - protein, 448 aa, Brassica oleracea
MAAAAMAVHLPKHSSFLTKPKHPSDQNSNFLGGSLKFGRSMSLNRKTKGPVMVSAASTVEGDRSKQFYINFTGFPFPLGPFLNRRTIRTEAVKGSIWMFEQEQALGFSSVSTNIRMTVIKLKSGGLWVHAPIAPTKECIQLIEELGAPVEYIVLPTFAYEHKIFVGPFSRKFPKAQVWVAPRQWSWPLNLPLEFFGIFRAKTIKDGDLSTPWADEIEQKVLSSPEVGIGPYVEVAFYHKRSRTLLVTDAVIFVPKKPPSSISSESLLASAKNGLAVKILSKGKQVPNDPVVDTPNTRQKGWERMVLQILFLGPSNLLEPNASFAQMSQKLIVSPIVKTLVFSKVPEKVRDWIDEIASDWRFKRIIPAHFEAPINAGRSEFLAAFGFLDDLLGERYVNRPPSLSVLFTSLMGKAASYFPPDDMRTLSSLDQFLVSVGAVKKTVSGRKRR

SEQ ID NO: 10 - protein, 395 aa, Brassica oleracea; identical to SEQ ID NO: 8

SEQ ID NO: 11 - protein, 326 aa, Brassica oleracea
MASSSQFRYTQTPSKVVHLRNLPWECVEEELIDLCKRFGKIVNTKTNVGANRNQAFVEFGDVNQAISMVSYYASSSEPAQIRGKTVYIQYSNRHEIVNNQSPGEVPGNVLLVTFEGVQSHHVCIDVIHLVFSAYGFVHKIATFEKAAGFQALVQFTDVDTALAARTALDGRSIPTYLLPEHVGSCNLRMSYSAHTDLNIKFQSHRSRDYTNPYLPVNQTAMDGSMQVFSAYGTVQKIAIFEKNGSTQALIQYSDIPTATIAKEALEGHCIYDGRLLDKSGDYTLPDLSQLVGQKVPGVAAASGPTDCWHNGQVQTQYTRSSYMYPL

SEQ ID NO: 12 - protein, 326 aa, Brassica oleracea; identical to SEQ ID NO: 11

SEQ ID NO: 13 - DNA, 19 bp, Artificial Sequence
  At3g01190 forward primer
ttcttccacgactgcttcg

SEQ ID NO: 14 - DNA, 21 bp, Artificial Sequence
  At3g01190 reverse primer
ctaacaaaactgatccgtcac

SEQ ID NO: 15 - DNA, 19 bp, Artificial Sequence
  At3g02420 forward primer
gttgcgttgccatctgcag

SEQ ID NO: 16 - DNA, 20 bp, Artificial Sequence
  At3g02420 reverse primer
caggctgagatagccattgg

SEQ ID NO: 17 - DNA, 20 bp, Artificial Sequence
  At3g07130 forward primer
ctactaaccatggagttacc

SEQ ID NO: 18 - DNA, 18 bp, Artificial Sequence
  At3g07130 reverse primer
aacgctggtgggattcac